European Patent Application EP 4 257 696 A2, published October 11, 2023. Title: Novel CRISPR DNA targeting enzymes and systems. Applicant: ARBOR BIOTECHNOLOGIES, INC. Application EP. The sequence listing filed with the application follows.

SEQUENCE LISTING (621 sequences)

SEQ ID NO: 1 - protein, 1046 aa, synthetic construct
  REGION 1..1046: note = Description of Artificial Sequence: Synthetic polypeptide
MVSESTIRPYTSKLAPNDPKLKMLNDTFNWLDHAYKVFFDVSVALFGAIEHETAQELIGEKSKFDADLLCAIMWFRLEEKSDNPGPLQTVEQRMRLFQKYSGHEPSSFTQEYIKGNIDSEKYQWVDCRLKFIDLARNINTTQESLKIDAYTLFMNKLIPVSKDDEFNAYGLISQLFGTGKKEDRSIKASMLEEISNIIEDKKPNTWEEYHDLIKKTFNVDNYKELKEKLSAGSSGRDSSLVIDLKEEKTGLLQPNFIKNRIVKFREDADKKRTVFLLPNRMKLREFIASQIGPFEQNSWSAVLNRSMAAIQSKNSSNILYTNEKEERNNEIQELLKKDILSAASILGDFRRGEFNRSVVSKNHLGARLNELFEIWQELTMDDGIKKYVDLCKDKFSRRPVKALLQYIYPYFDKINAKQFLDAASYNTLVETNNRKKIHPTVTGPTVCNWGPKSTINGSITPPNQMVKGRPAGSHGMIWVTMTVIDNGRWIKHHLPFHNSRYYEEHYCYREGLPTKNKPRTKQLGTQVGSTISAPSLAILKSQEEQDRRNDRKNRFKAHKSIIRSQENIEYNVAFDKSTNFDVTRKNGEFFITISSRVATPKYSYKLNIGDMIMGLDNNQTAPCTYSIWRVVEKDTEGSFFHNKIWLQLVTDGKVTSIVDNNRQVDQLSYAGIEYSNFAEWRKDRRQFLRSINEDYVKKSDNWRNMNLYQWNAEYSRLLLDVMKENKGKNIQNTFRAEIEELICGKFGIRLGSLFHHSLQFLTNCKSLISSYFMLNNKKEEYDQELFDSDFFRLMKSIGDKRVRKRKEKSSRISSTVLQIARENNVKSLCVEGYLPTSTKKTKPKQNQKSIDWCARAVVKKLNDGCKVLGINLQAIDPRDTSHLDPFVYYGKKSTKVGKEARYTIVEPSNIKEYMTNRFDDWHRGVTKKSKKGDVQTSTTVLLYQEALRQFASHYKLDFDSLPKMKFYELAKILGDHEKVIIPCRGGRAYLSTYPVTKDSSKITFNGRERWYNESDVVAAVNIVLRGIIDEDEQPDGAKKQALARTK

SEQ ID NO: 2 - protein, 1091 aa, synthetic construct
  REGION 1..1091: note = source = /note="Description of Artificial Sequence: Synthetic polypeptide"
MFTLLLSDISQQNFNKFLKNFFFTRNKTVVHCSSEIRHKGYRSNVMVSESTIRPYTSKLAPNDPKLKMLNDTFNWLDHAYKVFFDVSVALFGAIEHETAQELIGEKSKFDADLLCAIMWFRLEEKSDNPGPLQTVEQRMRLFQKYSGHEPSSFTQEYIKGNIDSEKYQWVDCRLKFIDLARNINTTQESLKIDAYTLFMNKLIPVSKDDEFNAYGLISQLFGTGKKEDRSIKASMLEEISNIIEDKKPNTWEEYHDLIKKTFNVDNYKELKEKLSAGSSGRDSSLVIDLKEEKTGLLQPNFIKNRIVKFREDADKKRTVFLLPNRMKLREFIASQIGPFEQNSWSAVLNRSMAAIQSKNSSNILYTNEKEERNNEIQELLKKDILSAASILGDFRRGEFNRSVVSKNHLGARLNELFEIWQELTMDDGIKKYVDLCKDKFSRRPVKALLQYIYPYFDKINAKQFLDAASYNTLVETNNRKKIHPTVTGPTVCNWGPKSTINGSITPPNQMVKGRPAGSHGMIWVTMTVIDNGRWIKHHLPFHNSRYYEEHYCYREGLPTKNKPRTKQLGTQVGSTISAPSLAILKSQEEQDRRNDRKNRFKAHKSIIRSQENIEYNVAFDKSTNFDVTRKNGEFFITISSRVATPKYSYKLNIGDMIMGLDNNQTAPCTYSIWRVVEKDTEGSFFHNKIWLQLVTDGKVTSIVDNNRQVDQLSYAGIEYSNFAEWRKDRRQFLRSINEDYVKKSDNWRNMNLYQWNAEYSRLLLDVMKENKGKNIQNTFRAEIEELICGKFGIRLGSLFHHSLQFLTNCKSLISSYFMLNNKKEEYDQELFDSDFFRLMKSIGDKRVRKRKEKSSRISSTVLQIARENNVKSLCVEGYLPTSTKKTKPKQNQKSIDWCARAVVKKLNDGCKVLGINLQAIDPRDTSHLDPFVYYGKKSTKVGKEARYTIVEPSNIKEYMTNRFDDWHRGVTKKSKKGDVQTSTTVLLYQEALRQFASHYKLDFDSLPKMKFYELAKILGDHEKVIIPCRGGRAYLSTYPVTKDSSKITFNGRERWYNESDVVAAVNIVLRGIIDEDEQPDGAKKQALARTK

SEQ ID NO: 3 - protein, 1093 aa, synthetic construct
  REGION 1..1093: note = source = /note="Description of Artificial Sequence: Synthetic polypeptide"
MSNKEKNASETRKAYTTKMIPRSHDRMKLLGNFMDYLMDGTPIFFELWNQFGGGIDRDIISGTANKDKISDDLLLAVNWFKVMPINSKPQGVSPSNLANLFQQYSGSEPDIQAQEYFASNFDTEKHQWKDMRVEYERLLAELQLSRSDMHHDLKLMYKEKCIGLSLSTAHYITSVMFGTGAKNNRQTKHQFYSKVIQLLEESTQINSVEQLASIILKAGDCDSYRKLRIRCSRKGATPSILKIVQDYELGTNHDDEVNVPSLIANLKEKLGRFEYECEWKCMEKIKAFLASKVGPYYLGSYSAMLENALSPIKGMTTKNCKFVLKQIDAKNDIKYENEPFGKIVEGFFDSPYFESDTNVKWVLHPHHIGESNIKTLWEDLNAIHSKYEEDIASLSEDKKEKRIKVYQGDVCQTINTYCEEVGKEAKTPLVQLLRYLYSRKDDIAVDKIIDGITFLSKKHKVEKQKINPVIQKYPSFNFGNNSKLLGKIISPKDKLKHNLKCNRNQVDNYIWIEIKVLNTKTMRWEKHHYALSSTRFLEEVYYPATSENPPDALAARFRTKTNGYEGKPALSAEQIEQIRSAPVGLRKVKKRQMRLEAARQQNLLPRYTWGKDFNINICKRGNNFEVTLATKVKKKKEKNYKVVLGYDANIVRKNTYAAIEAHANGDGVIDYNDLPVKPIESGFVTVESQVRDKSYDQLSYNGVKLLYCKPHVESRRSFLEKYRNGTMKDNRGNNIQIDFMKDFEAIADDETSLYYFNMKYCKLLQSSIRNHSSQAKEYREEIFELLRDGKLSVLKLSSLSNLSFVMFKVAKSLIGTYFGHLLKKPKNSKSDVKAPPITDEDKQKADPEMFALRLALEEKRLNKVKSKKEVIANKIVAKALELRDKYGPVLIKGENISDTTKKGKKSSTNSFLMDWLARGVANKVKEMVMMHQGLEFVEVNPNFTSHQDPFVHKNPENTFRARYSRCTPSELTEKNRKEILSFLSDKPSKRPTNAYYNEGAMAFLATYGLKKNDVLGVSLEKFKQIMANILHQRSEDQLLFPSRGGMFYLATYKLDADATSVNWNGKQFWVCNADLVAAYNVGLVDIQKDFKKK

SEQ ID NO: 4 - protein, 1033 aa, synthetic construct
  REGION 1..1033: note = source = /note="Description of Artificial Sequence: Synthetic polypeptide"
MMSDNIILPYNSKLAPDERKQRLLNDTFNWFDMCNEVFFDFVKNLYGGVKHEHLILVNFAEKPKKVSNSKKPKKKDQEVNIHVEPNQAEWVDNACATFWFRLQAKSTVQLDQSVQTAEERIRRFRDYAGHEPSSFAKSYLNGNYDPEKTEWVDCRLLYVNFCRNLNVNLDADIRTMVEHNLLPVLPGQDFKTNNVFSNIFGVGNKEDKGQKTNWLNTVSEGLQSKEIWNWDEYRDLISRSTGCSTAAELRSESIGRPSMLAVDFASEKSGQISQEWLAERVKSFRAAASQKSKIYDMPNRLVLKEYIASKIGPFKLERWSAAAVSAYKDVRSKNSINLLYSKERLWRCKEIAQILVDNTQVAEAQQILVNYSSGDTNSFTVENRHMGDLTVLFKIWEKMDMDSGIEQYSEIYRDEYSRDPITELLRYLYNHRHISAKTFRAAARLNSLLLKNDRKKIHPTISGRTSVSFGHSTIKGCITPPDHIVKNRKENAGSTGMIWVTMQLIDNGRWADHHIPFHNSRYYRDFYAYRADLPTISDPRRKSFGHRIGNNISDTRMINHDCKKASKMYLRTIQNMTHNVAFDQQTQFAVRRYADNNFTITIQARVVGRKYKKEISVGDRVMGVDQNQTTSNTYSVWEVVAEGTENSYPYKGNNYRLVEDGFIRSECSGRDQLSYDGLDFQDFAQWRRERYAFLSSVGCILNDEIEPQIPVSAEKAKKKKKFSKWRGCSLYSWNLCYAYYLKGLMHENLANNPAGFRQEILNFIQGSRGVRLCSLNHTSFRLLSKAKSLIHSFFGLNNIKDPESQRDFDPEIYDIMVNLTQRKTNKRKEKANRITSSILQIANRLNVSRIVIENDLPNASSKNKASANQRATDWCARNVSEKLEYACKMLGISLWQIDPRDTSHLDPFVVGKEARFMKIKVSDINEYTISNFKKWHANIATTSTTAPLYHDALKAFSSHYGIDWDNLPEMKFWELKNALKDHKEVFIPNRGGRCYLSTLPVTSTSEKIVFNGRERWLNASDIVAGVNIVLRSV

SEQ ID NO: 5 - protein, 1054 aa, synthetic construct
  REGION 1..1054: note = source = /note="Description of Artificial Sequence: Synthetic polypeptide"
MSSAIKSYKSVLRPNERKNQLLKSTIQCLEDGSAFFFKMLQGLFGGITPEIVRFSTEQEKQQQDIALWCAVNWFRPVSQDSLTHTIASDNLVEKFEEYYGGTASDAIKQYFSASIGESYYWNDCRQQYYDLCRELGVEVSDLTHDLEILCREKCLAVATESNQNNSIISVLFGTGEKEDRSVKLRITKKILEAISNLKEIPKNVAPIQEIILNVAKATKETFRQVYAGNLGAPSTLEKFIAKDGQKEFDLKKLQTDLKKVIRGKSKERDWCCQEELRSYVEQNTIQYDLWAWGEMFNKAHTALKIKSTRNYNFAKQRLEQFKEIQSLNNLLVVKKLNDFFDSEFFSGEETYTICVHHLGGKDLSKLYKAWEDDPADPENAIVVLCDDLKNNFKKEPIRNILRYIFTIRQECSAQDILAAAKYNQQLDRYKSQKANPSVLGNQGFTWTNAVILPEKAQRNDRPNSLDLRIWLYLKLRHPDGRWKKHHIPFYDTRFFQEIYAAGNSPVDTCQFRTPRFGYHLPKLTDQTAIRVNKKHVKAAKTEARIRLAIQQGTLPVSNLKITEISATINSKGQVRIPVKFDVGRQKGTLQIGDRFCGYDQNQTASHAYSLWEVVKEGQYHKELGCFVRFISSGDIVSITENRGNQFDQLSYEGLAYPQYADWRKKASKFVSLWQITKKNKKKEIVTVEAKEKFDAICKYQPRLYKFNKEYAYLLRDIVRGKSLVELQQIRQEIFRFIEQDCGVTRLGSLSLSTLETVKAVKGIIYSYFSTALNASKNNPISDEQRKEFDPELFALLEKLELIRTRKKKQKVERIANSLIQTCLENNIKFIRGEGDLSTTNNATKKKANSRSMDWLARGVFNKIRQLAPMHNITLFGCGSLYTSHQDPLVHRNPDKAMKCRWAAIPVKDIGDWVLRKLSQNLRAKNIGTGEYYHQGVKEFLSHYELQDLEEELLKWRSDRKSNIPCWVLQNRLAEKLGNKEAVVYIPVRGGRIYFATHKVATGAVSIVFDQKQVWVCNADHVAAANIALTVKGIGEQSSDEENPDGSRIKLQLTS

SEQ ID NO: 6 - DNA, 36 bp, synthetic construct
  misc_feature 1..36: note = source = /note="Description of Artificial Sequence: Synthetic oligonucleotide"
  source 1..36: mol_type = other DNA
cccacaatacctgagaaatccgtcctacgttgacgg

SEQ ID NO: 7 - DNA, 24 bp, synthetic construct
  misc_feature 1..24: note = source = /note="Description of Artificial Sequence: Synthetic oligonucleotide"
  source 1..24: mol_type = other DNA
aatttttgtgcccatcgttggcac

SEQ ID NO: 8 - DNA, 36 bp, synthetic construct
  misc_feature 1..36: note = source = /note="Description of Artificial Sequence: Synthetic oligonucleotide"
  source 1..36: mol_type = other DNA
ctctcaatgccttagaaatccgtccttggttgacgg

SEQ ID NO: 9 - DNA, 34 bp, synthetic construct
  misc_feature 1..34: note = source = /note="Description of Artificial Sequence: Synthetic oligonucleotide"
  source 1..34: mol_type = other DNA
gcaacacctaagaaatccgtctttcattgacggg

SEQ ID NO: 10 - DNA, 36 bp, synthetic construct
  misc_feature 1..36: note = source = /note="Description of Artificial Sequence: Synthetic oligonucleotide"
  source 1..36: mol_type = other DNA
gttgcaaaacccaagaaatccgtctttcattgacgg

SEQ ID NO: 11 - protein, 1080 aa, synthetic construct
  REGION 1..1080: note = source = /note="Description of Artificial Sequence: Synthetic polypeptide"
MPRNYFLGIFSLQKNKSVVHCSVEIRHKGYRSSVMVSDSTIRPYASKLAPNDPKLKMLNDTFNWLDHAYKVFFDVSVALFGAIEHETAQELIGEKSKFDADLICAIMWFRLEEKSDNPGPLQTVEQRMRLFQKYSGHEPSSFTQEYIKGNIDSEKYEWVDCRLKFIDLARNINTTQESLKIDAYTLFMNKLIPVSKDDEFNAYGLISQLFGTGKKEDRSIKAAMLEEISNILADKKPDTWEEYHDLIKKNFNVDNYKELKEKLSAGSSGRDSSLVIDLKEEKTGLLQPNFIKNRIVKFREDADKKKTVFLLPNRMKLREFIASQIGPFEQNSWSAVLNRSMAAIQSKNSSNILYTNEKEERNNEIQELLKKDILSAASILGDFRRGEFNRSVVSKNHLGARLNELFEIWQDLTMDDGIRKYVDLCKDKFSRRPVKALLQYIYPYFDKITAKQFLDAASYNTLVETNNRKKIHPTVTGPTVCNWGPKSTINGSITPPNQMVKGRPAGSHGMIWVTMTVIDNGRWIKHHLPFYNSRYYEEHYCYREGLPTKNQPRTKQLGTQVGSTISATSLAALKSQEEQDRRNDRKNRFKAHKSIIRSQENIEYNVAFDKSTNFDVTRKNGEFFITISSRVATPKYSYKLNIGDMIMGLDNNQTAPCTYSIWRVVEKDTEGSFFHNKIWLQLVTDGKITSIVDNNRQVDQLSYAGIEYSNFAEWRKDRRQFLRSINEDYVKKSDNWRNMNLYQWNAEYSRLLLDVMKENKGKNIQNTFRAEIEELICGKFGIRLGSLFHHSLQFLTNCKSLISSYFMLNNKKEEYDQELFDSDFFRLMKSIGDKRVRKRKEKSSRISSTVLQIARENNIKSLCVEGDLPTATKKTKPKQNQKSIDWCARAVVKKLNDGCKVLGINLQAIDPRDTSHLDPFVYYGKKSTKVGKEARYTIVEPSNIKEYMTNRFDDWHRGVTKKSKKGDVQTSTTVLLYQEALRQFASHYELDFDSLPKMKFYDLAKRLGDHEKVIIPCRGGRAYLSTYPVTKDSSKITFNGRERWYNESDVVAAVNIVLRGIRDEDEQPDDAKKQALARTK

SEQ ID NO: 12 - protein, 1046 aa, synthetic construct
  REGION 1..1046: note = source = /note="Description of Artificial Sequence: Synthetic polypeptide"
MVSDSTIRPYASKLAPNDPKLKMLNDTFNWLDHAYKVFFDVSVALFGAIEHETAQELIGEKSKFDADLICAIMWFRLEEKSDNPGPLQTVEQRMRLFQKYSGHEPSSFTQEYIKGNIDSEKYEWVDCRLKFIDLARNINTTQESLKIDAYTLFMNKLIPVSKDDEFNAYGLISQLFGTGKKEDRSIKAAMLEEISNILADKKPDTWEEYHDLIKKNFNVDNYKELKEKLSAGSSGRDSSLVIDLKEEKTGLLQPNFIKNRIVKFREDADKKKTVFLLPNRMKLREFIASQIGPFEQNSWSAVLNRSMAAIQSKNSSNILYTNEKEERNNEIQELLKKDILSAASILGDFRRGEFNRSVVSKNHLGARLNELFEIWQDLTMDDGIRKYVDLCKDKFSRRPVKALLQYIYPYFDKITAKQFLDAASYNTLVETNNRKKIHPTVTGPTVCNWGPKSTINGSITPPNQMVKGRPAGSHGMIWVTMTVIDNGRWIKHHLPFYNSRYYEEHYCYREGLPTKNQPRTKQLGTQVGSTISATSLAALKSQEEQDRRNDRKNRFKAHKSIIRSQENIEYNVAFDKSTNFDVTRKNGEFFITISSRVATPKYSYKLNIGDMIMGLDNNQTAPCTYSIWRVVEKDTEGSFFHNKIWLQLVTDGKITSIVDNNRQVDQLSYAGIEYSNFAEWRKDRRQFLRSINEDYVKKSDNWRNMNLYQWNAEYSRLLLDVMKENKGKNIQNTFRAEIEELICGKFGIRLGSLFHHSLQFLTNCKSLISSYFMLNNKKEEYDQELFDSDFFRLMKSIGDKRVRKRKEKSSRISSTVLQIARENNIKSLCVEGDLPTATKKTKPKQNQKSIDWCARAVVKKLNDGCKVLGINLQAIDPRDTSHLDPFVYYGKKSTKVGKEARYTIVEPSNIKEYMTNRFDDWHRGVTKKSKKGDVQTSTTVLLYQEALRQFASHYELDFDSLPKMKFYDLAKRLGDHEKVIIPCRGGRAYLSTYPVTKDSSKITFNGRERWYNESDVVAAVNIVLRGIRDEDEQPDDAKKQALARTK

SEQ ID NO: 13 - protein, 1046 aa, synthetic construct
  REGION 1..1046: note = source = /note="Description of Artificial Sequence: Synthetic polypeptide"
MVSESTIRPYTSKLAPNDSKLKMLNDTFNWLDHAYKVFFDVSVALFGAIEHETAQELIGEKSKFDADLLCAIMWFRLEEKSDNPGPLQTVEQRMRLFQKYSGHEPSSFTQEYIKGNIDSEKYQWVDCRLKFIDLARNINTTQESLKIDAYTLFMNKLIPVSKDDEFNAYGLISQLFGTGKKEDRSIKASMLEEISNILADKNPNTWEEYQDLIKKTFNVDNYKELKEKLSAGSSGRDGSLVIDLKEEKTGLLQPNFIKNRIVKFREDADKKRTVFLLPNRMKLREFIASQIGPFEQNSWSAVLNRSMAAIQSKNSSNILYTNEKEERNNEIQELLKKDILSAASILGDFRRGEFNRSVVSKNHLGARLNELFEIWQELTMDDGIKKYVDLCKDKFSRRPVKALLQYIYPYFDKINAKQFLDAASYNTLVETNNRKKIHPTVTGPTVCNWGPKSTINGSITPPNQMVKGRPAGSHGMIWVTMTVIDNGRWIKHHLPFHNSRYYEEHYCYREGLPTKNKPRTKQLGTQVGSTISAPSLAILKSQEEQDRRNDRKNRFKAHKSIIRSQENIEYNVAFDKSTNFDVTRKNGEFFITISSRVATPKYSYKLNIGDMIMGLDNNQTAPCTYSIWRVVEKDTEGSFFHNKIWLQLVTDGKVTSIVDNNRQVDQLSYAGIEYSNFAEWRKDRRQFLRSINEDYVKKSDNWRNMNLYQWNAEYSRLLLDVMKENKGKNIQNTFRAEIEELICGKFGIRLGSLFHHSLQFLTNCKSLISSYFMLNNKKEEYDQELFDSDFFRLMKSIGDKRVRKRKEKSSRISSTVLQIARENNVKSLCVEGYLPTSTKKTKPKQNQKSIDWCARAVVKKLNDGCKVLGIYLQAIDPRDTSHLDPFVYYGKKSTKVGKEARHTIVEPSNIKEYMTNRFDDWHRGVTKKSKKGDVQTSTTVLLYQEALRQFASHYKLDFDSLPKMKFYELAKILGDHEKVIIPCRGGRAYLSTYPVTKDSSKITFNGRERWYNESDVVAAVNIVLRGIIDEDEQPDGAKKQATTRRT

SEQ ID NO: 14 - protein, 1098 aa, synthetic construct
  REGION 1..1098: note = source = /note="Description of Artificial Sequence: Synthetic polypeptide"
MSISNNNILPYNPKLLPDDRKHKMLVDTFNQLDLIRNNLHDMIIALYGALKYDNIKQFASKEKPHISADALCSINWFRLVKTNERKPAIESNQIISKFIQYSGHTPDKYALSHITGNHEPSHKWIDCREYAINYARIMHLSFSQFQDLATACLNCKILILNGTLTSSWAWGANSALFGGSDKENFSVKAKILNSFIENLKDEMNTTKFQVVEKVCQQIGSSDAADLFDLYRSTVKDGNRGPATGRNPKVMNLFSQDGEISSEQREDFIESFQKVMQEKNSKQIIPHLDKLKYHLVKQSGLYDIYSWAAAIKNANSTIVASNSSNLNTILNKTEKQQTFEELRKDEKIVACSKILLSVNDTLPEDLHYNPSTSNLGKNLDVFFDLLNENSVHTIENKEEKNKIVKECVNQYMEECKGLNKPPMPVLLTFISDYAHKHQAQDFLSAAKMNFIDLKIKSIKVVPTVHGSSPYTWISNLSKKNKDGKMIRTPNSSLIGWIIPPEEIHDQKFAGQNPIIWAVLRVYCNNKWEMHHFPFSDSRFFTEVYAYKPNLPYLPGGENRSKRFGYRHSTNLSNESRQILLDKSKYAKANKSVLRCMENMTHNVVFDPKTSLNIRIKTDKNNSPVLDDKGRITFVMQINHRILEKYNNTKIEIGDRILAYDQNQSENHTYAILQRTEEGSHAHQFNGWYVRVLETGKVTSIVQGLSGPIDQLNYDGMPVTSHKFNCWQADRSAFVSQFASLKISETETFDEAYQAINAQGAYTWNLFYLRILRKALRVCHMENINQFREEILAISKNRLSPMSLGSLSQNSLKMIRAFKSIINCYMSRMSFVDELQKKEGDLELHTIMRLTDNKLNDKRVEKINRASSFLTNKAHSMGCKMIVGESDLPVADSKTSKKQNVDRMDWCARALSHKVEYACKLMGLAYRGIPAYMSSHQDPLVHLVESKRSVLRPRFVVADKSDVKQHHLDNLRRMLNSKTKVGTAVYYREAVELMCEELGIHKTDMAKGKVSLSDFVDKFIGEKAIFPQRGGRFYMSTKRLTTGAKLICYSGSDVWLSDADEIAAINIGMFVVCDQTGAFKKKKKEKLDDEECDILPFRPM

SEQ ID NO: 15 - protein, 1088 aa, synthetic construct
  REGION 1..1088: note = source = /note="Description of Artificial Sequence: Synthetic polypeptide"
MSSQVVRPYNAKFLPDDRKHKMLTDTINQLDKISSKHFDLLVAFYGSIQHKHVSINDKQEEHITPDSVCAINWFRPMSKDYAKYQVKIDSMITNFKEYAGHIPDKYAIEYMGSNIDTDRFVWVDCRNFAKDYVRNMDMSFSEFQNLVDALVFCKILALNESTSTNWAWGAISAIYGGGDKEDSQFKAKVLNTFVKALNDENNKTKFDVINKVCSDLGYNDHLSLIEDFRSTIDENGNKKSASGSPPAIAKFTEDGEISDNYRRACISSFSKTAKEKQDKKSIPHLDILKTHMIAMCGEYNTYAWTEAIKNANTDITSRNTRNMTFIKEKIESRNSLKIYDTEENMKAAKILNGINHKLTPDLHYTPAPKHLGKNLKDLFEMLEEKNILAQNEKEKKAALDECIKQYIDDCKGLNQQPIASLLAHISNYHKEITAENFLDGAKLLVLLQKINRQKAHPSVFSPKAYTWGSKLEKNRRAANSALLGWIVPPEEKHKDRHAGQHPVMWVTMTLLNNGKWEKHHVPFTNSRFFSEVYAYQPELPYKEGGYARNSKTATKPSQIMLPAYAESMRHHIATKGNGHKKSEKIVLRALSNIRHNVRFDPSTSFFVRIMRDKKGNHRLDTKGRITFGLQINHRITVGKTKSEINIGDRLLAFDQNQSENHTFAIMQRVEENTPNSHQFNGWNIRVLETGKVVSMTKGIESYYDQLSYDGVPYETKKFEDWRNERKAFVKKNKDIVIKEEKTFGQMFAEIKKSSLYKWNLSYLKILRMAIRAKSGDTVSLFREELISIAKNRFGPLGLGSLSASSLKMLGAFCGVIQSYFSVLNCLDDKDKSNFDSELYFYLVSAFEKRVFKRNEKTSRASSFIMAMAYNHGCKMIVCEDDLPTAGAGANKRQNSDRMDWCARSLAQKIKTGCEAMSIAYRAIPAYMSSHQDPLVHLADGKTSVLCPRFALVSKDDIKQYQLDGMRRMLNSKSKIGTAVYYRAAVELLCKELGINKTDIAKGKLSVSQFADIVNGEILLPQRGGRVYLATKELTNGAKLVSYNGSDVWLSNADEIAAINIGMFVVCTQTGVFGKKKKKDEQDGDIEIA

SEQ ID NO: 16 - protein, 1074 aa, synthetic construct
  REGION 1..1074: note = source = /note="Description of Artificial Sequence: Synthetic polypeptide"
MASISRPYGTKLRPDARKKEMLDKFFNTLTKGQRVFADLALCIYGSLTLEMAKSLEPESDSELVCAIGWFRLVDKTIWSKDGIKQENLVKQYEAYSGKEASEVVKTYLNSPSSDKYVWIDCRQKFLRFQRELGTRNLSEDFECMLFEQYIRLTKGEIEGYAAISNMFGNGEKEDRSKKRMYATRMKDWLEANENITWEQYREALKNQLNAKNLEQVVANYKGNAGGADPFFKYSFSKEGMVSKKEHAQQLDKFKTVLKNKARDLNFPNKEKLKQYLEAEIGIPVDANVYSQMFSNGVSEVQPKTTRNMSFSNEKLDLLTELKDLNKGDGFEYAREVLNGFFDSELHTTEDKFNITSRYLGGDKSNRLSKLYKIWKKEGVDCEEGIQQFCEAVKDKMGQIPIRNVLKYLWQFRETVSAEDFEAAAKANHLEEKISRVKAHPIVISNRYWAFGTSALVGNIMPADKRHQGEYAGQNFKMWLEAELHYDGKKAKHHLPFYNARFFEEVYCYHPSVAEITPFKTKQFGCEIGKDIPDYVSVALKDNPYKKATKRILRAIYNPVANTTGVDKTTNCSFMIKRENDEYKLVINRKISVDRPKRIEVGRTIMGYDRNQTASDTYWIGRLVPPGTRGAYRIGEWSVQYIKSGPVLSSTQGVNNSTTDQLVYNGMPSSSERFKAWKKARMAFIRKLIRQLNDEGLESKGQDYIPENPSSFDVRGETLYVFNSNYLKALVSKHRKAKKPVEGILDEIEAWTSKDKDSCSLMRLSSLSDASMQGIASLKSLINSYFNKNGCKTIEDKEKFNPVLYAKLVEVEQRRTNKRSEKVGRIAGSLEQLALLNGVEVVIGEADLGEVEKGKSKKQNSRNMDWCAKQVAQRLEYKLAFHGIGYFGVNPMYTSHQDPFEHRRVADHIVMRARFEEVNVENIAEWHVRNFSNYLRADSGTGLYYKQATMDFLKHYGLEEHAEGLENKKIKFYDFRKILEDKNLTSVIIPKRGGRIYMATNPVTSDSTPITYAGKTYNRCNADEVAAANIVISVLAPRSKKNEEQDDIPLITKKAESKSPPKDRKRSKTSQLPQK

SEQ ID NO: 17 - protein, 1031 aa, synthetic construct
  REGION 1..1031: note = source = /note="Description of Artificial Sequence: Synthetic polypeptide"
MVSDSTIRPYTSKLAPNDPKRKMLNDTFNWLDHAYKVFFDVSVALFGGIDYEAAEELIDEKSTFDADLLCAIMWFRLEEKSNNPGPLQTTEQRTRLFQKYSGHEPSSFAQEYIKGNTDTEKYEWVDCRLKFADLARNIHTTQESLKTDAYTLFMNKLIPVSKDDEFNAYGFISQLFGTGKKEDRSVKASMLEEISNIIEDKKPNTWEEYQDLIKKTFNVSNYKELKEKLSAGSSGRDGSLVIDLKEEKTGLLQPNFIKNRIVKFREDADKKRTVFSLPNRMKLREFISSQIGPFEQNSWSAVLNRSMAAIQSKNSSNILYTNQKQERNNEIQELLKEDILSAASILNDFRRGEFNSSVVSKNHLGSRLNELFEMWQALKMNDGIEKYTDLCKDNFSRRPVSALLQYIYPYFDKITAKQFLDAASYNTLVETNNRKKIHPTVTGPTVCNWGPKSTINGSITPPNQMVKDRPAGSHGMIWVTMTVRDNGRWVKHHLPFHNSRYYEEHYCYREGLPTKNQPRTKQLGTQVGSIISAPSLAILKSQEEQDRRNDRKSRFKAHKSIIRSQENIKYNVAFDKSTNFDVTRKNGEFFITISSRVTTPKYSHKLNVGDIIMGLDNNQTAPCTYSIWRIVEKDTEGSFFHNKIWLQLVTDGKITSIVDNNRQVDQLSYAGVEYSNFAEWRKDRRQFLRSINEDYVKKSDNWLNMNLYQWNAEYSRLLLGVMKDNKDKNIQNTFRAEIEELICGKFGIRLGSLSHHSLQFLTNCKSLISSYFMLNNKKEEHDQESFDSDFFRLMRSIDDKRIRKRKEKSSRISSSVLQIARENNVKSLCVEGDLPTATKKTKPKQNQKSIDWCARAVVKKLNDGCKVLGINLQAIDPRDTSHLDPFVYYGKKSTKVGKEARYVIVEPSNIKEYMTKKFTDWHRGVSKKSKKGDVQTSTTAPLYQEALKQFADHYKLDFDSLPKMKFYELAKILEDHKQVIIPCRGGRAYLSTYPITKDSSKINFNGRERWYNQSDVVAAVNIVLRGIRDEN

SEQ ID NO: 18 - protein, 1066 aa, synthetic construct
  REGION 1..1066: note = source = /note="Description of Artificial Sequence: Synthetic polypeptide"
MPDPIKSYKSPIIIDPNNAHDVEKLDFLRETFVYLSNGTKCFMHVFLSLLGGMNETLAKKIVSLETPKKEKKKKSNKPSHKIELFLAICWFRLVKISKNESSVLPALLGNRFEKYFGAKATPEVMEYFSANYDEATYAWKDMREEFVSLKSKLKVSEKDLISDIGSMINERYIGLKFGKPWGIISGLFGEGKKVDRSLKVELLKNVLEEIEKNPPKTKDQLAKMILKCADCKNGQEIHAKCGKIGRMSSVSNWADEVGSEKEIVLSFVKSKISQDLAKQSNERNWKCVNALKSYILSEIGNCFDQSSWSEMLNNSLSVIQSKTTRNYNFCIEQLEEKKNLNQNHRKFGTMIEDYFSSRFFTGENKFIICNFHVGDKDKVSALLASCEGLSEEELEEKIQNFCESQKQESKMPIPALLMYLNSLKDSITVDQMFQGILYNKIRDKIERQKLHPIVPNNDSFDWGMSSKINGRIISPKEKAKHNAQNNRSLYDSGIWIEISVLKNKEWAKHHYKISNTRFVEEFYYPSSNDENSLDQVFRTGRNGFNNPAKNNLSLEQVSNIKNAPKNRRRAIKRQMRVEAAHQQNVLPHVKWDDNYCITISKYGDKFVTFISKKFKSKKSKEYVVFLGFDQNQTASHTFAAVQICDSKDENVIPYCGLFVKPLECGHITSVQKVKDRSIDQLSYSGLPWKDFISWSQERKEFVSKWRMVEVKTRNGEKLDDLTVKINKLDENKHGLYAYNSKYFWYLKSIMRKKTKDELFEIRKELLTVIKTGRLCVLRLSSLNHSSFLMLKNAKSAISCYFNNLLKGVSNDQEKYEADPEMFELRREVEAKRQNKCMSKKNLISSQIVSKAIELRGNYGSVAIIGEDLSDYVPDKGKKSTQNANLLDWLSRGVANKVKQIANMHDNISFKDVSPQWTSHQDSFVDRNPNSALRVRFGSCDPEEMYEKDFESLIKFLKEDCGHYTNSMNDFLSHYGVSRKDMLEIKFSAFKILMKNILNKTGEKSLLYPKRGGRLYLATHKLGQCTRRTYNGVDFWECDADCVAAFNIALSGIRKYYGIKSEAVSPV

SEQ ID NO: 19 - DNA, 36 bp, synthetic construct
  misc_feature 1..36: note = source = /note="Description of Artificial Sequence: Synthetic oligonucleotide"
  source 1..36: mol_type = other DNA
ctagcaatgacctaatagtgtgtccttagttgacat

SEQ ID NO: 20 - DNA, 36 bp, synthetic construct
  misc_feature 1..36: note = source = /note="Description of Artificial Sequence: Synthetic oligonucleotide"
  source 1..36: mol_type = other DNA
tctcaacgatagtcagacatgtgtcctcagtgacac

SEQ ID NO: 21 - DNA, 36 bp, synthetic construct
  misc_feature 1..36: note = source = /note="Description of Artificial Sequence: Synthetic oligonucleotide"
  source 1..36: mol_type = other DNA
cctacaatacctaagaaatccgtcctaagttgacgg

SEQ ID NO: 22 - DNA, 37 bp, synthetic construct
  misc_feature 1..37: note = source = /note="Description of Artificial Sequence: Synthetic oligonucleotide"
  source 1..37: mol_type = other DNA
gtagcaatcagtacatattgtgcctttcattggcaca

SEQ ID NO: 23 - DNA, 36 bp, synthetic construct
  misc_feature 1..36: note = source = /note="Description of Artificial Sequence: Synthetic oligonucleotide"
  source 1..36: mol_type = other DNA
gtagcaatcagtacatattgtgcctttcattggcac

SEQ ID NO: 24 - DNA, 36 bp, synthetic construct
  misc_feature 1..36: note = source = /note="Description of Artificial Sequence: Synthetic oligonucleotide"
  source 1..36: mol_type = other DNA
gttggaatgactaatttttgtgcccaccgttggcac

SEQ ID NO: 25-99 - skipped (75 entries)

SEQ ID NO: 100 - RNA, 23 nt, synthetic construct
  misc_feature 1..23: note = source = /note="Description of Artificial Sequence: Synthetic oligonucleotide"
  source 1..23: mol_type = other RNA
atttttgtgcccatcgttggcac

SEQ ID NO: 101 - RNA, 23 nt, synthetic construct
  misc_feature 1..23: note = source = /note="Description of Artificial Sequence: Synthetic oligonucleotide"
  source 1..23: mol_type = other RNA
agaaatccgtctttcattgacgg

SEQ ID NO: 102-149 - skipped (48 entries)

SEQ ID NO: 150 - RNA, 106 nt, synthetic construct
  variation 37..70: note = a, c, u, g, unknown or other
  misc_feature 1..106: note = source = /note="Description of Artificial Sequence: Synthetic polynucleotide"
  source 1..106: mol_type = other RNA
ctagcaatgacctaatagtgtgtccttagttgacatnnnnnnnnnnnnnnnnnnnnnnnnnnnnnnnnnnctagcaatgacctaatagtgtgtccttagttgacat

SEQ ID NO: 151 - RNA, 107 nt, synthetic construct
  variation 37..71: note = a, c, u, g, unknown or other
  misc_feature 1..107: note = source = /note="Description of Artificial Sequence: Synthetic polynucleotide"
  source 1..107: mol_type = other RNA
ctagcaatgacctaatagtgtgtccttagttgacatnnnnnnnnnnnnnnnnnnnnnnnnnnnnnnnnnnnctagcaatgacctaatagtgtgtccttagttgacat

SEQ ID NO: 152 - RNA, 108 nt, synthetic construct
  variation 37..72: note = a, c, u, g, unknown or other
  misc_feature 1..108: note = source = /note="Description of Artificial Sequence: Synthetic polynucleotide"
  source 1..108: mol_type = other RNA
tctcaacgatagtcagacatgtgtcctcagtgacacnnnnnnnnnnnnnnnnnnnnnnnnnnnnnnnnnnnntctcaacgatagtcagacatgtgtcctcagtgacac

SEQ ID NO: 153 - RNA, 107 nt, synthetic construct
  variation 37..71: note = a, c, u, g, unknown or other
  misc_feature 1..107: note = source = /note="Description of Artificial Sequence: Synthetic polynucleotide"
  source 1..107: mol_type = other RNA
cctacaatacctaagaaatccgtcctaagttgacggnnnnnnnnnnnnnnnnnnnnnnnnnnnnnnnnnnncctacaatacctaagaaatccgtcctaagttgacgg

SEQ ID NO: 154 - RNA, 107 nt, synthetic construct
  variation 38..70: note = a, c, u, g, unknown or other
  misc_feature 1..107: note = source = /note="Description of Artificial Sequence: Synthetic polynucleotide"
  source 1..107: mol_type = other RNA
gtagcaatcagtacatattgtgcctttcattggcacannnnnnnnnnnnnnnnnnnnnnnnnnnnnnnnngtagcaatcagtacatattgtgcctttcattggcaca

SEQ ID NO: 155 - RNA, 106 nt, synthetic construct
  variation 37..70: note = a, c, u, g, unknown or other
  misc_feature 1..106: note = source = /note="Description of Artificial Sequence: Synthetic polynucleotide"
  source 1..106: mol_type = other RNA
gtagcaatcagtacatattgtgcctttcattggcacnnnnnnnnnnnnnnnnnnnnnnnnnnnnnnnnnngtagcaatcagtacatattgtgcctttcattggcac

SEQ ID NO: 156 - RNA, 108 nt, synthetic construct
  variation 37..72: note = a, c, u, g, unknown or other
  misc_feature 1..108: note = source = /note="Description of Artificial Sequence: Synthetic polynucleotide"
  source 1..108: mol_type = other RNA
gttggaatgactaatttttgtgcccaccgttggcacnnnnnnnnnnnnnnnnnnnnnnnnnnnnnnnnnnnngttggaatgactaatttttgtgcccaccgttggcac

SEQ ID NO: 157 - RNA, 84 nt, synthetic construct
  variation 25..60: note = a, c, u, g, unknown or other
  misc_feature 1..84: note = source = /note="Description of Artificial Sequence: Synthetic oligonucleotide"
  source 1..84: mol_type = other RNA
aatttttgtgcccatcgttggcacnnnnnnnnnnnnnnnnnnnnnnnnnnnnnnnnnnnnaatttttgtgcccatcgttggcac

SEQ ID NO: 158 - RNA, 108 nt, synthetic construct
  variation 37..72: note = a, c, u, g, unknown or other
  misc_feature 1..108: note = source = /note="Description of Artificial Sequence: Synthetic polynucleotide"
  source 1..108: mol_type = other RNA
cccacaatacctgagaaatccgtcctacgttgacggnnnnnnnnnnnnnnnnnnnnnnnnnnnnnnnnnnnncccacaatacctgagaaatccgtcctacgttgacgg

SEQ ID NO: 159 - RNA, 108 nt, synthetic construct; identical to SEQ ID NO: 158
  variation 37..72: note = a, c, u, g, unknown or other
  misc_feature 1..108: note = source = /note="Description of Artificial Sequence: Synthetic polynucleotide"
  source 1..108: mol_type = other RNA

SEQ ID NO: 160 - RNA, 108 nt, synthetic construct
  variation 37..72: note = a, c, u, g, unknown or other
  misc_feature 1..108: note = source = /note="Description of Artificial Sequence: Synthetic polynucleotide"
  source 1..108: mol_type = other RNA
ctctcaatgccttagaaatccgtccttggttgacggnnnnnnnnnnnnnnnnnnnnnnnnnnnnnnnnnnnnctctcaatgccttagaaatccgtccttggttgacgg

SEQ ID NO: 161 - RNA, 106 nt, synthetic construct
  variation 37..70: note = a, c, u, g, unknown or other
  misc_feature 1..106: note = source = /note="Description of Artificial Sequence: Synthetic polynucleotide"
  source 1..106: mol_type = other RNA
cccacaatacctgagaaatccgtcctacgttgacggnnnnnnnnnnnnnnnnnnnnnnnnnnnnnnnnnncccacaatacctgagaaatccgtcctacgttgacgg

SEQ ID NO: 162 - RNA, 92 nt, synthetic construct
  variation 35..58: note = a, c, u, g, unknown or other
  misc_feature 1..92: note = source = /note="Description of Artificial Sequence: Synthetic oligonucleotide"
  source 1..92: mol_type = other RNA
gcaacacctaagaaatccgtctttcattgacgggnnnnnnnnnnnnnnnnnnnnnnnngcaacacctaagaaatccgtctttcattgacggg

SEQ ID NO: 163 - RNA, 103 nt, synthetic construct
  variation 37..67: note = a, c, u, g, unknown or other
  misc_feature 1..103: note = source = /note="Description of Artificial Sequence: Synthetic polynucleotide"
  source 1..103: mol_type = other RNA
gttgcaaaacccaagaaatccgtctttcattgacggnnnnnnnnnnnnnnnnnnnnnnnnnnnnnnngttgcaaaacccaagaaatccgtctttcattgacgg

SEQ ID NO: 164-199 - skipped (36 entries)

SEQ ID NO: 200 - protein, 7 aa, synthetic construct
  VARIANT 1: note = /replace="Thr"
  VARIANT 4: note = /replace="Leu"
  VARIANT 6: note = /replace="Ser"
  VARIANT 7: note = /replace="Leu"
  SITE 1..7: note = /note="Variant residues given in the sequence have no preference with respect to those in the annotations for variant positions"
  REGION 1..7: note = source = /note="Description of Artificial Sequence: Synthetic peptide"
SSHQDPF

SEQ ID NO: 201 - protein, 11 aa, synthetic construct
  VARIANT 1: note = /replace="Gly" or "Ser"
  MOD_RES 2: note = Any amino acid
  MOD_RES 4: note = Any amino acid
  VARIANT 6: note = /replace="Ile"
  VARIANT 7: note = /replace="Ser" or "Val"
  MOD_RES 8..10: note = Any amino acid
  VARIANT 11: note = /replace="Ala"
  SITE 1..11: note = /note="Variant residues given in the sequence have no preference with respect to those in the annotations for variant positions"
  REGION 1..11: note = source = /note="Description of Artificial Sequence: Synthetic peptide"
AXDXNQTXXXT

SEQ ID NO: 202 - RNA, 17 nt, synthetic construct
  variation 6..11: note = a, c, u, g, unknown or other
  misc_feature 1..17: note = source = /note="Description of Artificial Sequence: Synthetic oligonucleotide"
  source 1..17: mol_type = other RNA
ccgtcnnnnnntgacgg

SEQ ID NO: 203 - RNA, 17 nt, synthetic construct
  variation 6..11: note = a, c, u, g, unknown or other
  misc_feature 1..17: note = source = /note="Description of Artificial Sequence: Synthetic oligonucleotide"
  source 1..17: mol_type = other RNA
gtgccnnnnnntggcac

SEQ ID NO: 204 - RNA, 17 nt, synthetic construct
  variation 6..11: note = a, c, u, g, unknown or other
  misc_feature 11: note = May or may not be present
  misc_feature 1..17: note = source = /note="Description of Artificial Sequence: Synthetic oligonucleotide"
  source 1..17: mol_type = other RNA
gtgtcnnnnnntgacay

SEQ ID NO: 205 - RNA, 14 nt, synthetic construct
  misc_feature 1..14: note = source = /note="Description of Artificial Sequence: Synthetic oligonucleotide"
  source 1..14: mol_type = other RNA
tcytwvrttgacgg

SEQ ID NO: 206 - RNA, 14 nt, synthetic construct
  misc_feature 1..14: note = source = /note="Description of Artificial Sequence: Synthetic oligonucleotide"
  source 1..14: mol_type = other RNA
ccywycrttggcac

SEQ ID NO: 207-209 - skipped (3 entries)

SEQ ID NO: 210 - protein, 4 aa, synthetic construct
  VARIANT 1: note = /replace="Phe" or "Ile" or "Leu" or "Met" or "Pro" or "Val" or "Trp" or "Tyr"
  VARIANT 2: note = /replace="Phe" or "Ile" or "Leu" or "Met" or "Pro" or "Arg" or "Val" or "Trp" or "Tyr"
  VARIANT 3: note = /replace="Phe" or "Gly" or "Ile" or "Leu" or "Met" or "Pro" or "Val" or "Trp" or "Tyr"
  SITE 1..4: note = /note="Variant residues given in the sequence have no preference with respect to those in the annotations for variant positions"
  REGION 1..4: note = source = /note="Description of Artificial Sequence: Synthetic peptide"
CCCE

SEQ ID NO: 211-299 - skipped (89 entries)

SEQ ID NO: 300 - protein, 7 aa, Simian virus 40
PKKKRKV

SEQ ID NO: 301 - protein, 16 aa, unidentified
  REGION 1..16: note = source = /note="Description of Unknown: Nucleoplasmin bipartite NLS sequence"
KRPAATKKAGQAKKKK

SEQ ID NO: 302 - protein, 9 aa, unidentified
  REGION 1..9: note = source = /note="Description of Unknown: c-Myc NLS sequence"
PAAKRVKLD

SEQ ID NO: 303 - protein, 11 aa, unidentified
  REGION 1..11: note = source = /note="Description of Unknown: c-Myc NLS sequence"
RQRRNELKRSP

SEQ ID NO: 304 - protein, 38 aa, Homo sapiens
NQSSNFGPMKGGNFGGRSSGPYGGGGQYFAKPRNQGGY

SEQ ID NO: 305 - protein, 42 aa, unidentified
  REGION 1..42: note = source = /note="Description of Unknown: IBB domain from importin-alpha sequence"
RMRIZFKNKGKDTAELRRRRVEVSVELRKAKKDEQILKRRNV

SEQ ID NO: 306 - protein, 8 aa, unidentified
  REGION 1..8: note = source = /note="Description of Unknown: Myoma T protein sequence"
VSRKRPRP

SEQ ID NO: 307 - protein, 8 aa, unidentified
  REGION 1..8: note = source = /note="Description of Unknown: Myoma T protein sequence"
PPKKARED

SEQ ID NO: 308 - protein, 8 aa, Homo sapiens
PQPKKKPL

SEQ ID NO: 309 - protein, 12 aa, Mus sp.
SALIKKKKKMAP

SEQ ID NO: 310 - protein, 5 aa, Influenza virus
DRLRR

SEQ ID NO: 311 - protein, 7 aa, Influenza virus
PKQKKRK

SEQ ID NO: 312 - protein, 10 aa, Hepatitis virus
RKLKKKIKKL

SEQ ID NO: 313 - protein, 10 aa, Mus sp.
REKKKFLKRR

SEQ ID NO: 314 - protein, 20 aa, Homo sapiens
KRKGDEVDGVDEVAKKKSKK

SEQ ID NO: 315 - protein, 17 aa, Homo sapiens
RKCLQAGMNLEARKTKK

SEQ ID NO: 316-399 - skipped (84 entries)

SEQ ID NO: 400 - RNA, 131 nt, synthetic construct
  misc_feature 1..131: note = source = /note="Description of Artificial Sequence: Synthetic polynucleotide"
  source 1..131: mol_type = other RNA
gggaatttttgtgcccatcgttggcaccctaatgcggaagtagtgggtaacccggaatttttgtgcccatcgttggcactccgcaagaattgattggctccaattctaatttttgtgcccatcgttggcac

SEQ ID NO: 401 - RNA, 24 nt, synthetic construct
  misc_feature 1..24: note = source = /note="Description of Artificial Sequence: Synthetic oligonucleotide"
  source 1..24: mol_type = other RNA
aatttttgtgcccatcgttggcac

SEQ ID NO: 402 - RNA, 28 nt, synthetic construct
  misc_feature 1..28: note = source = /note="Description of Artificial Sequence: Synthetic oligonucleotide"
  source 1..28: mol_type = other RNA
cctaatgcggaagtagtgggtaacccgg

SEQ ID NO: 403 - RNA, 28 nt, synthetic construct
  misc_feature 1..28: note = source = /note="Description of Artificial Sequence: Synthetic oligonucleotide"
  source 1..28: mol_type = other RNA
tccgcaagaattgattggctccaattct

SEQ ID NO: 404 - RNA, 131 nt, synthetic construct
  misc_feature 1..131: note = source = /note="Description of Artificial Sequence: Synthetic polynucleotide"
  source 1..131: mol_type = other RNA
gggaatttttgtgcccatcgttggcacaggcatcatcagcattaaccacgcaaacaatttttgtgcccatcgttggcacgcgtgctggattgcttcgatggtctgcgaatttttgtgcccatcgttggcac

SEQ ID NO: 405 - RNA, 24 nt, synthetic construct
  misc_feature 1..24: note = source = /note="Description of Artificial Sequence: Synthetic oligonucleotide"
  source 1..24: mol_type = other RNA
aatttttgtgcccatcgttggcac

SEQ ID NO: 406 - RNA, 28 nt, synthetic construct
  misc_feature 1..28: note = source = /note="Description of Artificial Sequence: Synthetic oligonucleotide"
  source 1..28: mol_type = other RNA
aggcatcatcagcattaaccacgcaaac

SEQ ID NO: 407 - RNA, 28 nt, synthetic construct
  misc_feature 1..28: note = source = /note="Description of Artificial Sequence: Synthetic oligonucleotide"
  source 1..28: mol_type = other RNA
gcgtgctggattgcttcgatggtctgcg

SEQ ID NO: 408 - DNA, 128 bp, synthetic construct
  misc_feature 1..128: note = source = /note="Description of Artificial Sequence: Synthetic polynucleotide"
  source 1..128: mol_type = other DNA
catgtggaccacattaggctgcaaaactgcgcatttacgaaaacgcgaaagtttgcgtggttaatgctgatgatgccttaacaatgccgattcgcggtgcggatgaacgtaatttctcgaggcgtatt

SEQ ID NO: 409 - DNA, 128 bp, synthetic construct
  misc_feature 1..128: note = source = /note="Description of Artificial Sequence: Synthetic polynucleotide"
  source 1..128: mol_type = other DNA
catgtggaccacattaggcttggttgttgctgccgacgacggtgtgatgccgcagaccatcgaagcaatccagcacgcgaaagcggcgcaggtaccggtggtggttgcgtaatttctcgaggcgtatt

SEQ ID NO: 410 - DNA, 128 bp, synthetic construct
  misc_feature 1..128: note = source = /note="Description of Artificial Sequence: Synthetic polynucleotide"
  source 1..128: mol_type = other DNA
aatacgcctcgagaaattacaaagtgatgcaggcgtttccaggtgctttccctaatgcggaagtagtgggtaacccggtgcgtaccgatgtgttggcgctgccgttgcagcctaatgtggtccacatg

SEQ ID NO: 411 - DNA, 171 bp, synthetic construct
  misc_feature 1..171: note = source = /note="Description of Artificial Sequence: Synthetic polynucleotide"
  source 1..171: mol_type = other DNA
gtgccaacgatgggcacaaaaattagaattggagccaatcaattcttgcggagtgccaacgatgggcacaaaaattagaattggagccaatcaattcttgcggagtgccaacgatgggcacaaaaattccctatagtgagtcgtattactcgagggatccttattacattt

SEQ ID NO: 412 - DNA, 18 bp, synthetic construct
  misc_feature 1..18: note = source = /note="Description of Artificial Sequence: Synthetic primer"
  source 1..18: mol_type = other DNA
taatacgactcactatag

SEQ ID NO: 413 - DNA, 52 bp, synthetic construct
  misc_feature 1..52: note = source = /note="Description of Artificial Sequence: Synthetic primer"
  source 1..52: mol_type = other DNA
gtgccaacgatgggcacaaaaattagaattggagccaatcaattcttgcgga

SEQ ID NO: 414 - DNA, 171 bp, synthetic construct
  misc_feature 1..171: note = source = /note="Description of Artificial Sequence: Synthetic polynucleotide"
  source 1..171: mol_type = other DNA
gtgccaacgatgggcacaaaaattcgcagaccatcgaagcaatccagcacgcgtgccaacgatgggcacaaaaattgtttgcgtggttaatgctgatgatgcctgtgccaacgatgggcacaaaaattccctatagtgagtcgtattactcgagggatccttattacattt

SEQ ID NO: 415 - DNA, 18 bp, synthetic construct
  misc_feature 1..18: note = source = /note="Description of Artificial Sequence: Synthetic primer"
  source 1..18: mol_type = other DNA
taatacgactcactatag

SEQ ID NO: 416 - DNA, 52 bp, synthetic construct
  misc_feature 1..52: note = source = /note="Description of Artificial Sequence: Synthetic primer"
  source 1..52: mol_type = other DNA
gtgccaacgatgggcacaaaaattcgcagaccatcgaagcaatccagcacgc

SEQ ID NO: 417-499 - skipped (83 entries)

SEQ ID NO: 500 - DNA, 212 bp, synthetic construct
  misc_feature 1..212: note = source = /note="Description of Artificial Sequence: Synthetic polynucleotide"
  source 1..212: mol_type = other DNA
gggcagagcgcacatcgcccacagtccccgagaagttggggggaggggtcggcaattgatccggtgcctagagaaggtggcgcggggtaaactgggaaagtgatgtcgtgtactggctccgcctttttcccgagggtgggggagaaccgtatataagtgcagtagtcgccgtgaacgttctttttcgcaacgggtttgccgccagaacacag

SEQ ID NO: 501 - DNA, 3375 bp, synthetic construct
  misc_feature 1..3375: note = source = /note="Description of Artificial Sequence: Synthetic polynucleotide"
  source 1..3375: mol_type = other DNA
atgaaaatcgaagaaggtaaaggtcaccatcaccatcaccacatgtctaacaaggagaagaatgccagcgagacccggaaggcctacaccacaaagatgatccccaggagccacgaccgcatgaagctgctgggcaactttatggactatctgatggatggcacccctatcttctttgagctgtggaatcagttcggcggcggcatcgacagagatatcatcagcggcacagccaacaaggataagatctccgacgatctgctgctggccgtgaactggtttaaagtgatgccaatcaattctaagccccagggcgtgtccccttctaacctggccaatctgttccagcagtacagcggatccgagcctgacatccaggcacaggagtatttcgcctccaactttgacaccgagaagcaccagtggaaggatatgcgggtggagtacgagagactgctggccgagctgcagctgtctaggagcgacatgcatcacgatctgaagctgatgtacaaggagaagtgcatcggcctgtccctgtctaccgcccactatatcacaagcgtgatgtttggcaccggcgccaagaacaatcgccagacaaagcaccagttctattccaaagtgatccagctgctggaggagagcacccagatcaattccgtggagcagctggcctccatcatcctgaaggccggcgactgcgattcttacaggaagctgaggatcaggtgttcccgcaagggagcaaccccatctatcctgaagatcgtgcaggactatgagctgggcacaaaccacgacgatgaagtgaatgtgccctccctgatcgccaacctgaaggagaagctgggcaggtttgagtacgagtgcgagtggaagtgtatggagaagatcaaggccttcctggcctctaaagtgggcccttactatctgggcagctattccgccatgctggagaatgccctgagcccaatcaagggcatgaccacaaagaactgtaagttcgtgctgaagcagatcgacgccaagaacgatatcaagtacgagaatgagccctttggcaagatcgtggagggcttctttgactctccttatttcgagagcgataccaatgtgaagtgggtgctgcaccctcaccacatcggcgagtctaacatcaagacactgtgggaggacctgaatgccatccacagcaagtacgaggaggacatcgcctctctgagcgaggataagaaggagaagcggatcaaggtgtaccagggcgatgtgtgccagaccatcaacacatattgtgaggaagtgggcaaggaggccaagaccccactggtgcagctgctgaggtacctgtattcccgcaaggacgatatcgccgtggacaagatcatcgatggcatcacattcctgtctaagaagcacaaggtggagaagcagaagatcaacccagtgatccagaagtaccccagcttcaattttggcaacaattccaagctgctgggcaagatcatcagcccaaaggacaagctgaagcacaacctgaagtgcaacagaaatcaggtggataattacatctggatcgagatcaaggtgctgaacaccaagacaatgcggtgggagaagcaccactatgccctgagctccaccagatttctggaggaggtgtactatcccgccacatccgagaatccacctgacgcactggcagcacggttcagaaccaagacaaacggctacgagggcaagccagccctgtctgccgagcagatcgagcagatcaggagcgcaccagtgggactgagaaaggtgaagaagcggcagatgagactggaggcagcaaggcagcagaatctgctgccacgctatacctggggcaaggattttaacatcaatatctgtaagaggggcaacaatttcgaggtgaccctggccacaaaggtgaagaagaagaaggagaagaactacaaggtggtgctgggctatgacgccaacatcgtgcgcaagaatacctacgcagcaatcgaggcacacgcaaacggcgatggcgtgatcgactataatgatctgcctgtgaagccaatcgagtctggctttgtgacagtggagagccaggtgagggacaagtcctacgatcagctgtcttataacggcgtgaagctgctgtactgcaagcctcacgtggagagccggagatccttcctggagaagtatcggaacggcaccatgaaggacaatagaggcaacaatatccagatcgacttcatgaaggattttgaggccatcgccgacgatgagacaagcctgtactacttcaacatgaagtactgtaagctgctgcagtctagcatccgcaaccactcctctcaggccaaggagtatagggaggagatcttcgagctgctgcgcgatggcaagctgtccgtgctgaagctgagctccctgtctaatctgagcttcgtgatgtttaaggtggccaagtctctgatcggcacctactttggccacctgctgaagaagcctaagaactccaagtctgacgtgaaggccccacccatcacagacgaggataagcagaaggccgatccagagatgttcgcactgcggctggcactggaggagaagagactgaataaggtgaagagcaagaaggaagtgatcgccaacaagatcgtggccaaggcactggagctgagggacaagtacggaccagtgctgatcaagggcgagaatatcagcgataccacaaagaagggcaagaagtctagcaccaattccttcctgatggactggctggccagaggcgtggccaacaaggtgaaggagatggtcatgatgcaccagggcctggagttcgtggaggtgaaccccaattttacctcccaccaggatcctttcgtgcacaagaacccagagaataccttccgggcaaggtacagcaggtgcaccccttccgagctgacagagaagaaccgcaaggagatcctgtccttcctgtctgacaagcccagcaagcggcctactaacgcctactataatgagggcgccatggcctttctggccacatatggcctgaagaagaatgacgtgctgggcgtgtccctggagaagttcaagcagatcatggccaacatcctgcaccagcggtccgaggatcagctgctgtttccctctagaggcggcatgttctacctggccacctataagctggacgccgatgccacaagcgtgaactggaatggcaagcagttttgggtgtgtaacgccgacctggtggccgcctacaatgtgggcctggtggacatccagaaggatttcaagaagaagaaaaggccggcggccacgaaaaaggccggccaggcaaaaaagaaaaagtaataa

SEQ ID NO: 502 - DNA, 3258 bp, synthetic construct
  misc_feature 1..3258: note = source = /note="Description of Artificial Sequence: Synthetic polynucleotide"
  source 1..3258: mol_type = other DNA
atgaaaatcgaagaaggtaaaggtcaccatcaccatcaccacatgagctccgccatcaagtcctacaagtctgtgctgcggccaaacgagagaaagaatcagctgctgaagagcaccatccagtgcctggaggacggctccgccttctttttcaagatgctgcagggcctgtttggcggcatcacccccgagatcgtgagattcagcacagagcaggagaagcagcagcaggatatcgccctgtggtgtgccgtgaattggttcaggcctgtgagccaggactccctgacccacacaatcgcctccgataacctggtggagaagtttgaggagtactatggcggcacagccagcgacgccatcaagcagtacttcagcgcctccatcggcgagtcctactattggaatgactgccgccagcagtactatgatctgtgtcgggagctgggcgtggaggtgtctgacctgacccacgatctggagatcctgtgccgggagaagtgtctggccgtggccacagagagcaaccagaacaattctatcatcagcgtgctgtttggcaccggcgagaaggaggataggtctgtgaagctgcgcatcacaaagaagatcctggaggccatcagcaacctgaaggagatcccaaagaatgtggcccccatccaggagatcatcctgaatgtggccaaggccaccaaggagacattcagacaggtgtacgcaggaaacctgggagcaccatccaccctggagaagtttatcgccaaggacggccagaaggagttcgatctgaagaagctgcagacagacctgaagaaagtgatccggggcaagtctaaggagagagattggtgctgtcaggaggagctgaggagctacgtggagcagaataccatccagtatgacctgtgggcctggggcgagatgttcaacaaggcccacaccgccctgaagatcaagtccacaagaaactacaattttgccaagcagaggctggagcagttcaaggagatccagtctctgaacaatctgctggtggtgaagaagctgaacgactttttcgatagcgagtttttctccggcgaggagacctacacaatctgcgtgcaccacctgggcggcaaggacctgtccaagctgtataaggcctgggaggacgatcccgccgatcctgagaatgccatcgtggtgctgtgcgacgatctgaagaacaattttaagaaggagcctatcaggaacatcctgcgctacatcttcaccatccgccaggagtgtagcgcacaggacatcctggcagcagcaaagtacaatcagcagctggatcggtataagagccagaaggccaacccatccgtgctgggcaatcagggctttacctggacaaacgccgtgatcctgccagagaaggcccagcggaacgacagacccaattctctggatctgcgcatctggctgtacctgaagctgcggcaccctgacggcagatggaagaagcaccacatcccattctacgatacccggtttttccaggagatctatgccgccggcaatagccctgtggacacctgtcagtttaggacaccccgcttcggctatcacctgcctaagctgaccgatcagacagccatccgcgtgaacaagaagcacgtgaaggcagcaaagaccgaggcacggatcagactggccatccagcagggcacactgccagtgtccaatctgaagatcaccgagatctccgccacaatcaactctaagggccaggtgcgcatccccgtgaagtttgacgtgggaaggcagaagggaaccctgcagatcggcgaccggttctgcggctacgatcagaaccagacagcctctcacgcctatagcctgtgggaggtggtgaaggagggccagtaccacaaggagctgggctgttttgtgcgcttcatctctagcggcgacatcgtgtccatcaccgagaaccggggcaatcagtttgatcagctgtcttatgagggcctggcctacccccagtatgccgactggagaaagaaggcctccaagttcgtgtctctgtggcagatcaccaagaagaacaagaagaaggagatcgtgacagtggaggccaaggagaagtttgacgccatctgcaagtaccagcctaggctgtataagttcaacaaggagtacgcctatctgctgcgggatatcgtgagaggcaagagcctggtggagctgcagcagatcaggcaggagatctttcgcttcatcgagcaggactgtggagtgacccgcctgggatctctgagcctgtccaccctggagacagtgaaggccgtgaagggcatcatctactcctatttttctacagccctgaatgcctctaagaacaatcccatcagcgacgagcagcggaaggagtttgatcctgagctgttcgccctgctggagaagctggagctgatcaggactcggaagaagaagcagaaggtggagagaatcgccaatagcctgatccagacatgcctggagaacaatatcaagttcatcaggggcgagggcgacctgtccaccacaaacaatgccaccaagaagaaggccaactctaggagcatggattggctggccagaggcgtgtttaataagatccggcagctggccccaatgcacaacatcaccctgttcggctgcggcagcctgtacacatcccaccaggaccctctggtgcacagaaacccagataaggccatgaagtgtagatgggcagcaatcccagtgaaggacatcggcgattgggtgctgagaaagctgtcccagaacctgagggccaagaatatcggcaccggcgagtactatcaccagggcgtgaaggagttcctgtctcactatgagctgcaggacctggaggaggagctgctgaagtggcggtctgatagaaagagcaacatcccttgctgggtgctgcagaatagactggccgagaagctgggcaacaaggaggccgtggtgtacatcccagtgaggggcggccgcatctattttgcaacccacaaggtggcaacaggagccgtgagcatcgtgttcgaccagaagcaagtgtgggtgtgtaatgcagatcacgtggcagcagcaaacatcgcactgaccgtgaagggcatcggcgagcagtcctctgacgaggagaaccccgatggctccaggatcaagctgcagctgacatctaaaaggccggcggccacgaaaaaggccggccaggcaaaaaagaaaaagtaataa

SEQ ID NO: 503 - DNA, 228 bp, synthetic construct
  misc_feature 1..228: note = source = /note="Description of Artificial Sequence: Synthetic polynucleotide"
  source 1..228: mol_type = other DNA
cgactgtgccttctagttgccagccatctgttgtttgcccctcccccgtgccttccttgaccctggaaggtgccactcccactgtcctttcctaataaaatgaggaaattgcatcgcattgtctgagtaggtgtcattctattctggggggtggggtggggcaggacagcaagggggaggattgggaagacaatagcaggcatgctggggatgcggtgggctctatgg

SEQ ID NO: 504-549 - skipped (46 entries)

SEQ ID NO: 550 - DNA, 45 bp, synthetic construct
  misc_feature 1..45: note = source = /note="Description of Artificial Sequence: Synthetic oligonucleotide"
  source 1..45: mol_type = other DNA
accccctttccaaagcccattccctcttttcgagccggggtgtgc

SEQ ID NO: 551 - DNA, 45 bp, synthetic construct
  misc_feature 1..45: note = source = /note="Description of Artificial Sequence: Synthetic oligonucleotide"
  source 1..45: mol_type = other DNA
accccctttccaaagcccattccctctttttgagccggggtgtgc

SEQ ID NO: 552 - DNA, 45 bp, synthetic construct
  misc_feature 1..45: note = source = /note="Description of Artificial Sequence: Synthetic oligonucleotide"
  source 1..45: mol_type = other DNA
accccctttccaaagcccattccctgtttatgagccggggtgtgc

SEQ ID NO: 553 - DNA, 44 bp, synthetic construct
  misc_feature 1..44: note = source = /note="Description of Artificial Sequence: Synthetic oligonucleotide"
  source 1..44: mol_type = other DNA
accccctttccaaagcccattccctctttaagagccggggtgtg

SEQ ID NO: 554 - DNA, 44 bp, synthetic construct
  misc_feature 1..44: note = source = /note="Description of Artificial Sequence: Synthetic oligonucleotide"
  source 1..44: mol_type = other DNA
accccctttccaaagcccattacctctttaagagccggggtgtg

SEQ ID NO: 555 - DNA, 44 bp, synthetic construct
  misc_feature 1..44: note = source = /note="Description of Artificial Sequence: Synthetic oligonucleotide"
  source 1..44: mol_type = other DNA
accccctttccaaagcccattccctctgtaagagccggggtgtg

SEQ ID NO: 556-600 - skipped (45 entries)

SEQ ID NO: 601 - protein, 7 aa, synthetic construct
  REGION 1..7: note = source = /note="Description of Artificial Sequence: Synthetic peptide"
GSGGGGS

SEQ ID NO: 602 - protein, 15 aa, synthetic construct
  REGION 1..15: note = source = /note="Description of Artificial Sequence: Synthetic peptide"
GGGGSGGGGSGGGGS

SEQ ID NO: 603 - protein, 18 aa, synthetic construct
  REGION 1..18: note = source = /note="Description of Artificial Sequence: Synthetic peptide"
GGSGGSGGSGGSGGSGGS

SEQ ID NO: 604 - protein, 32 aa, synthetic construct
  REGION 1..32: note = source = /note="Description of Artificial Sequence: Synthetic polypeptide"
SGGSSGGSSGSETPGTSESATPESSGGSSGGS

SEQ ID NO: 605 - protein, 167 aa, synthetic construct
  REGION 1..167: note = source = /note="Description of Artificial Sequence: Synthetic polypeptide"
MSEVEFSHEYWMRHALTLAKRAWDEREVPVGAVLVHNNRVIGEGWNRPIGRHDPTAHAEIMALRQGGLVMQNYRLIDATLYVTLEPCVMCAGAMIHSRIGRVVFGARDAKTGAAGSLMDVLHHPGMNHRVEITEGILADECAALLSDFFRMRRQEIKAQKKAQSSTD

SEQ ID NO: 606 - protein, 167 aa, synthetic construct; identical to SEQ ID NO: 605
  REGION 1..167: note = source = /note="Description of Artificial Sequence: Synthetic polypeptide"

SEQ ID NO: 607 - protein, 198 aa, synthetic construct [sequence omitted]

SEQ ID NO: 608 - protein, 208 aa, synthetic construct
  REGION 1..208: note = source = /note="Description of Artificial Sequence: Synthetic polypeptide"
MTDAEYVRIHEKLDIYTFKKQFFNNKKSVSHRCYVLFELKRRGERRACFWGYAVNKPQSGTERGIHAEIFSIRKVEEYLRDNPGQFTINWYSSWSPCADCAEKILEWYNQELRGNGHTLKIWACKLYYEKNARNQIGLWNLRDNGVGLNVMVSEHYQCCRKIFIQSSHNQLNENRWLEKTLKRAEKRRSELSIMIQVKILHTTKSPAV

SEQ ID NO: 609 - protein, 229 aa, synthetic construct [sequence omitted]

SEQ ID NO: 610 - protein, 4 aa, unidentified
  REGION 1..4: note = source = /note="Description of Unknown: KDEL motif sequence"
KDEL

SEQ ID NO: 611 - protein, 5 aa, synthetic construct
  REGION 1..5: note = source = /note="Description of Artificial Sequence: Synthetic peptide"
EAAAK

SEQ ID NO: 612 - DNA, 44 bp, synthetic construct
  variation 24..44: note = a, c, u, g, unknown or other
  misc_feature 1..44: note = source = /note="Description of Artificial Sequence: Synthetic oligonucleotide"
  source 1..44: mol_type = other DNA
atttttgtgcccatcgttggcacnnnnnnnnnnnnnnnnnnnnn

SEQ ID NO: 613 - RNA, 44 nt, synthetic construct
  variation 24..44: note = a, c, u, g, unknown or other
  misc_feature 1..44: note = source = /note="Description of Artificial Sequence: Synthetic oligonucleotide"
  source 1..44: mol_type = other RNA
agaaatccgtctttcattgacggnnnnnnnnnnnnnnnnnnnnn

SEQ ID NO: 614 - DNA, 36 bp, synthetic construct
  misc_feature 1..36: note = source = /note="Description of Artificial Sequence: Synthetic oligonucleotide"
  source 1..36: mol_type = other DNA
ttcgcgtgctggattgcttcgatggtctgcggcatc

SEQ ID NO: 615 - DNA, 36 bp, synthetic construct
  misc_feature 1..36: note = source = /note="Description of Artificial Sequence: Synthetic oligonucleotide"
  source 1..36: mol_type = other DNA
gatgccgcagaccatcgaagcaatccagcacgcgaa

SEQ ID NO: 616 - RNA, 28 nt, synthetic construct
  misc_feature 1..28: note = source = /note="Description of Artificial Sequence: Synthetic oligonucleotide"
  source 1..28: mol_type = other RNA
gcgtgctggattgcttcgatggtctgcg

SEQ ID NO: 617 - RNA, 34 nt, synthetic construct
  misc_feature 1..34: note = source = /note="Description of Artificial Sequence: Synthetic oligonucleotide"
  source 1..34: mol_type = other RNA
gcaacacctaagaaatccgtctttcattgacggg

SEQ ID NO: 618 - RNA, 36 nt, synthetic construct
  misc_feature 1..36: note = source = /note="Description of Artificial Sequence: Synthetic oligonucleotide"
  source 1..36: mol_type = other RNA
gttgcaaaacccaagaaatccgtctttcattgacgg

SEQ ID NO: 619 - RNA, 24 nt, synthetic construct
  misc_feature 1..24: note = source = /note="Description of Artificial Sequence: Synthetic oligonucleotide"
  source 1..24: mol_type = other RNA
aatttttgtgcccatcgttggcac

SEQ ID NO: 620 - RNA, 36 nt, synthetic construct
  misc_feature 1..36: note = source = /note="Description of Artificial Sequence: Synthetic oligonucleotide"
  source 1..36: mol_type = other RNA
ctctcaatgccttagaaatccgtccttggttgacgg

SEQ ID NO: 621 - RNA, 36 nt, synthetic construct
  misc_feature 1..36: note = source = /note="Description of Artificial Sequence: Synthetic oligonucleotide"
  source 1..36: mol_type = other RNA
cccacaatacctgagaaatccgtcctacgttgacgg